European Patent Application EP 4 393 500 A1, published July 3, 2024. Title: 戈氏梭菌联合肿瘤血管生成抑制剂的应用. Applicant: 山东新创生物科技有限公司. The sequence listing filed with the application follows.

SEQUENCE LISTING (2 sequences)

SEQ ID NO: 1 - DNA, 25 bp, synthetic construct
  source 1..25: mol_type = other DNA
aatacagggaattttagaggtgcag

SEQ ID NO: 2 - DNA, 23 bp, synthetic construct
  source 1..23: mol_type = other DNA
gctaacatcttacaaggcccaca